European Patent Specification EP 3 676 278 B1, published April 12, 2023. Title: CYCLIC DINUCLEOTIDES AS ANTICANCER AGENTS. Applicant: BRISTOL-MYERS SQUIBB COMPANY. The sequence listing filed with the application follows.

SEQUENCE LISTING (2 sequences)

SEQ ID NO: 1 - protein, 210 aa, Artificial Sequence
  Homosapien
MGSSHHHHHHSSGETVRFQGHMSVAHGLAWSYYIGYLRLILPELQARIRTYNQHYNNLLRGAVSQRLYILLPLDCGVPDNLSMADPNIRFLDKLPQQTGDRAGIKDRVYSNSIYELLENGQRAGTCVLEYATPLQTLFAMSQYSQAGFSREDRLEQAKLFCRTLEDILADAPESQNNCRLIAYQEPADDSSFSLSQEVLRHLRQEEKEEV

SEQ ID NO: 2 - protein, 210 aa, Artificial Sequence
  Homosapien
MGSSHHHHHHSSGETVRFQGHMSVAHGLAWSYYIGYLRLILPELQARIRTYNQHYNNLLRGAVSQRLYILLPLDCGVPDNLSMADPNIRFLDKLPQQTADRAGIKDRVYSNSIYELLENGQRAGTCVLEYATPLQTLFAMSQYSQAGFSREDRLEQAKLFCQTLEDILADAPESQNNCRLIAYQEPADDSSFSLSQEVLRHLRQEEKEEV